European Patent Application EP 4 331 673 A1, published March 6, 2024. Title: Strip-shaped aggregate of retinal pigment epithelial cells, production device thereof and a production method of strip-shaped aggregate of retinal pigment epithelial cells using the device. Applicant: RIKEN. The sequence listing filed with the application follows.

SEQUENCE LISTING (10 sequences)

SEQ ID NO: 1 - DNA, 19 bp, Artificial Sequence
  primer
tagaaccatcagcgccgtc

SEQ ID NO: 2 - DNA, 21 bp, Artificial Sequence
  primer
tgagtgtagtgtgtatgttgg

SEQ ID NO: 3 - DNA, 20 bp, Artificial Sequence
  primer
tccccaatacaactgccact

SEQ ID NO: 4 - DNA, 20 bp, Artificial Sequence
  primer
ccttggcattcagaatcagg

SEQ ID NO: 5 - DNA, 20 bp, Artificial Sequence
  primer
gagggtgcaagagaaggaca

SEQ ID NO: 6 - DNA, 20 bp, Artificial Sequence
  primer
tgcagaagccattgatttga

SEQ ID NO: 7 - DNA, 20 bp, Artificial Sequence
  primer
tccttggccatcagaaaaag

SEQ ID NO: 8 - DNA, 20 bp, Artificial Sequence
  primer
catttgggtggctgaagtct

SEQ ID NO: 9 - DNA, 20 bp, Artificial Sequence
  primer
accacagtccatgccatcac

SEQ ID NO: 10 - DNA, 20 bp, Artificial Sequence
  primer
tccaccaccctgttgctgta